European Patent Application EP 4 681 722 A1, published January 21, 2026. Title: METHODS FOR THE TREATMENT OF INFLAMMATORY SKIN DISEASES WITH UROCANASE INHIBITOR. Applicant: INSERM. The sequence listing filed with the application follows.

SEQUENCE LISTING (4 sequences)

SEQ ID NO: 1 - protein, 552 aa, Bacillus subtilis
MTDVKKSIRANRGTELECLGWEQEAVLRMLRNNLDPEVAEKPEDLIVYGGIGKAARDWDAFHAIEHSLKTLKNDETLLVQSGKPVGMFRTHPQAPRVLLANSVLVPKWADWEHFHELEKKGLMMYGQMTAGSWIYIGSQGILQGTYETFAELARQHFGGSLKGTLTLTAGLGGMGGAQPLSVTMNEGVVIAVEVDEKRIDKRIETKYCDRKTASIEEALAWAEEAKLAGKPLSIALLGNAAEVHHTLLNRGVKIDIVTDQTSAHDPLIGYVPEGYSLDEADRLRQDTPELYVRLAKQSMKKHVEAMLAFQQKGSIVFDYGNNIRQVAKDEGLENAFDFPGFVPAYIRPLFCEGKGPFRWAALSGDPADIYRTDALLKELFPTNKALHRWIDMAQEKVTFQGLPSRICWLGYGERKKMGLAINELVRTGELKAPVVIGRDHLDCGSVASPNRETEAMKDGSDAVGDWAVLNALVNTAAGASWVSFHHGGGVGMGYSLHAGMVAVADGSELADERLARVLTSDPGMGIIRHADAGYERAVEVAKEQDIIVPMQK

SEQ ID NO: 2 - DNA, 28954 bp, Bacillus subtilis
  source 1..28954: mol_type = genomic DNA
aagcttccgcaagccgcatatcaaattgatgtgcctgccaaagaagcgggtgtcgtctctgaaatcgtcgcggacgaaatcggcgtcgcggcgatgctgttaggtgccggccgcgccacaaaagaagacgaaatcgatttagccgtcggatcatgctccgcaaaaaggtcggcgacaaagtagaaaaaggggaaccgctcgtaacgctttacgctaaccgagaaaacgtcgatgaagtcatcgcaaaagtctatgacaacatccgcatcgccgcggaagaagcgccgaagctgattcatacgttaattacagaataaaaaataaagcacatcccatgctgagcggggtgtgcttttttaattataggatgtgatcggctggatattcctcttggctgatttttttcgcttttgtaacatttcttttgaaatggtagatgagatagcaaaggatgatacaaggaactccgcagaaaagtgcgattctttgattgggatcaaaagcaagaccgatacaagaagcagaacataataagagagcggctataggcataagaggataaagcggcgtgcgaaatgtcagatcttttacatcccccccttttttcaaaaatctctttcgaaacaagagttgggacaaggcaatgctcatccagaccacgactcctgcaaatccagcaattgcgaccatcaccacatagacagttccaggggccacgatactggaaacgagagataaacaagatacagccatactgatcattaaggcatttaaaggaatgcctttagatgtcactttcttaaaacgggagctgatcatgttttcatttgctaaagaccacatcatacgggtcgaagcatataagcctgagttggcgacagacagcaaggctgttaatattacgaaattcataatatcagcagcgtaaggaattccgatctccgcaaatacggcgacaaacgggctttcaatcacgcctgcgtccttccatgaaatcaacccggataatatgaagacagcgccaatgaaaaaaatcacggttctccatgcgacattacggatggatcgcggtatatccttttgaggatttgctgattctcctgctgtaacgccgattaactctgtaccggaaaaggcgaagctcacagatatcatcgcgataaaaacggcgagaaagccatttggaaacaacccgccatgatctgtgaagtttgacaacataggagcatccgccgttccgtttaaagagatcaggccaaacatggcggctcctcctaaaatgataaataaaataatggtgacaatctttacgctggaaaaccaaaattcagtttccgcaaataacttaactgaaaatgcgttgcatataaaaagaagggctgcaaaaatcgcactccacatccatacactgctgtcagggaaccagcgctgcatgagaataccggatgcggtaaactcagagcctaccgtcaccacccaattgatccagtacatgatgccgaccataaaaccggtagatggaccgataaatgttgtagcatatttttgaaaagagccggtcaccgcattggcaaccgacaattcgccgagacattgcatgacgaggtacatcatcaacccgccgattacataagcgagtatcgtaccgccgggtccggcttgatgtagcgtatagcccgtactgaggaaaagtcctgtgcctatgacgcctcccaatgagatcataaataggtgcctgcttttcattgtgcgttttagctgttggctgctgttctcctgaagattcactgtctcgccctccttttagctgccattccttaggcagatgagtttcttatacccaaaatacaacctgccagaagatcacttgaatggggagagtttcattccttttaatgcgtgtaacagaacatgagctgcagctctgcttgtcatatctcgaaaatcgagggtagggtcgacttcaacaatttcaatcccggcaacattgggctgttgtgcgatgtacttgactgcttcaagcaattcgtctgtatagaggccgcccgggccaatcgctggacagccgggtgcatgggactggtctaagacatccatgtcaacagatataaaaatgaaatctgttttatcttgaacaacaggcaaaatctcttttatcgttgggattagtcctttttcccggatcatgtccatcgtgtgaatgttcacgttatgtttttttgcatatgcttcataggcctggctgttgctgaattctctgatacccagctggatcaaatgttgaccttcaatgatctcttcatccaaaaggcggcggaagggggtgccgtttgtcggccccccgtcctccgtattgcgaacatcgtgatgggcatcaaattgaatcaccgctgtcgttccttttgtttgtgctatcgcttttattgtggagtagctgatagagttatctcccccaagtatgagcggcacccaatccggatgatccgaaagcagagcgtgcatggtttggaaaatgtgatgatgtgactttacgatatcagtgacatgaatatcgatatcccccaggtcatatagaagctctgatacgacgtgctctccaagctcagcagaataggctgatgaatgtttcagagcctggcgtattgttccgggtgcaaaggaagcgcctgaatgactgatggaggattttgatagggggacacctatcaacgccggtcccttaatgtcctggccgtcccatgttgcgatcaggtcgctcatttttgtgacatcccggtctttaaacgaagatccggcctctctgagaaaagggtacttatccaagaatggctccctccctgttgacaacaattgttccatttttcatgacttgatgtacatgattgaccccgtagtgatacggaatatacatatagttcggggcttgccaaatgacaagatcagctgagcggccagctttgagctgaccggcttcttctccttttcctatggcatatgcggcattgactgtgaccgcgtgccatatttcttctgcagtcattttcagatgaagcgcggcaatggacataatcagctggatattttcagtcggcgagctgccaggattaaaatccgttgccaagctgacacatacaccttcatcaatcatagctcttgccctggcgtatgtgcttttgccaagataaaatgtcgtgcccggcaagaggacggcgatcgttcctgcctcagccaatttctttatgccttcgtccgatgtacctaccaaatggtcggctgagacggcctttagcttacctgctaattcagcacctccaagcggatcgatttcatctgcgtgtatttttaatccgaagcctgcctcagctgctttttgtaaataacggcgggattggctgactgtaaaaacgcctgtttctgtaaaaatatcagcaaagctggcgagctcctgctctttgatttccggcaaaagggaaagcatttgatccagaaaatcatctggatcgttttgatattcgggaggaatcgcatgggctcccataaatgtggaaacaaggtcaacaggctggctttcatgcagtttctttgcgacacgcaactgtttgagctctgtctctttttccaagccgtagccgcttttcacttctgctgtggttgtgccgtaggacagcattctttgcagatgaaaatgggctttttgcagcagctcttcttctgaagccgccctggtatccttgactgtagacagaatcccgccgccctgcgccagaatatccaaatatgaaatgccctgaagcttaaggttcatctccttttcacgagatccgccaaatacaagatgggtgtgcggatcaacgaggccaggcgttacaaggcgtcccgaacagtcaatgatttcgtctgcctcgtaaccggcttcagcccctttttgtccggcgaacacaattttctgttcatggatgccgacaacagcgtcttcgatcacatgaagatcctgcatgcttttgcctgcccgcggaccgctgctttccatcgtcaaaagctgaccgatgttgatgagaatcgtatcaatttgctttggcatgtcatcactcctttatttttgcatcggcacgataatgtcctgttccttcgctacttcaacggcacgttcataacccgcatccgcatgacggataatgcccattcctgggtcgctcgttaagacccgcgcgagccgctcgtcagccagctcacttccatcggccactgcaaccatgccggcatgaagggaatagcccattccgacgccgccgccatggtggaaggaaacccagcttgcacccgccgccgtgttgacaagcgcatttagcacagcccaatcaccgacagcgtcacttccatccttcatcgcttctgtttcccggtttggagaggcgacagacccgcagtccaaatgatctctcccaataacgacaggcgcttttagctccccggttctaaccagctcgttaatggcgaggcccatcttttttcgttctccatatccaagccagcagatacgggacggcaagccttggaaggtgactttttcctgtgccatatcaatccagcggtgaagggctttatttgtcgggaacagctcttttaataacgcatccgtacggtaaatatctgccggatctccggaaagcgccgcccagcggaacggcccttttccttcacagaataaggggcggatgtaggcagggacaaaccccggaaaatcgaaggcattctccagcccttcatcctttgcgacttgccggatattgttgccgtagtcaaatacaatagagcccttttgctgaaaggccagcatggcttcgacatgttttttcatgctttgcttcgcaaggcgcacgtaaagctctggagtgtcttgacgcaaacggtcagcttcatcaagggaatagccctcgggaacataaccgattaaagggtcatgggcagatgtctgatctgtcacaatatcaattttgacgcctcggttcaaaagtgtgtgatgcacctcagctgcgtttccgagaagtgcaatggacaaaggttttcctgccagctttgcctcttcagcccaagctaaggcttcctcaatcgatgctgtttttcgatcgcagtattttgtttcgatccgcttgtcgatgcgtttctcgtcaacctcgacggcaatcacgacgccttcattcatcgtgactgacagcggctgggcgcctcccattccgccgagacccgctgtcagcgtcaacgttccttttaagctgcccccgaagtgctgtcgcgccagctcagcgaaggtttcataggttccttgcaatatgccttgtgagccaatgtaaatccagctgccagccgtcatctgtccgtacatcattaacccttttttctcaagttcgtggaaatgctcccagtctgcccacttcggaacaagaacagaatttgctaggagcacgcgaggggcctgcgggtgtgtacggaacatgccaacgggctttccggattgcacgagcaatgtttcatcattttttaatgttttcaaggaatgctcaatggcgtgaaaagcgtcccaatcccgtgcggctttgccaatcccgccatatacgatgaggtcctccggcttctcggcgacttctggatcaaggttgtttcgaagcatccgaagcactgcctcttgctcccatcctaagcattcaagctctgttcctctgttggcacggattgatttttttacatcagtcatatgttcatcccccttagttctttattctgatgatcaggtattaaagattctttcttcagccagtcagtcaagcgttcaatgtcataggaaaaaacacggtcctgctgaatggacggcacgacttttctcatttcttgaaaaagctgtttcgtataggacgctgcatgttctatgcctctgtattcaacagcctgcaatgcgcaaatggcttcgatcgcaatgactctccttgtatttgcgatcacctgataagcatgccgagcggcgatggttcccatgctgacatggtcctcttggttggcggatgacggaatggaatccacacttgcaggatgggccagtgttttattttcagaaacgagtgaggccgcggcgtactgcatgatcattgcaccggattgcagaccgggatgagggctcaggaacggcggcaggtcattcagctgcggattcacaagtcgttcgatcctacgctctgcgatattcgcaagctctgatattgcgattttcagaaaatccatggcaaaggcgattggctgtccgtgaaagtttccgccggaaatcactttgtcaccgtcattgaaaatgagtggattgtctgtagctgcgttcatttcaatctctaatttttctttgacatatcctagtgtctgccaagtcgcaccgtgtacttgcggaatacagcgcaatgaataggcatcctgtacccgcagttctccctgggaggttgtcaggccgctgtcagatagataaaagcgaattcgttctgcgacatcgatctgctcctgatagccgcgggctaagtgaatatcctcgtcaaatgcatcgataattccctgcaacccctcaatcgttaagctggcaattcgttctgtttgataggctagtttctcagcttcgatgtaggcgaccacccccattgcagtcatggcctgagtcccgttaatcaaggcaagcccttccttggatgtcagcgttaccggttgaatacctgcttttttcaagcctgtcattgccggcattctttccccctcaaaaaagacttctccttgtccgatcagcgcaagcgccaagtgggaaagcggcgccagatctccgcttgcgccaagtgatccttgctgagggatgacaggatggacgcgtttatttaaaaaagcaagcaactgctcgatcagctcagcgcgtacaccggaaaagccttttaacagcgcattggcgcgcaaaagcagcattgccctggaaacacactcaggaaaagggtcgccgactccgcaggcatgagaaaggattaaattcagctgcagcgccgccgagtcttctttctgaatcaggacatcgctgaatttgccaaatccggtgttgatgccgtagattgtcttttcgtcgcgtacaatccgttccactgctgctctgctttttttcacgcgctccatactttcctcagaagccgctgcctcctcaaaatcaaacagcacacgagcgacgtcggctgttgtcaatgaagaaccgtctaaagtcaccataagcccaactcctttttctttactttggtaaagcgcccatacaaaaaggagctatgctgtgaacttctgttttcacgcatagccccctatcgtctaagatctatgggctgtttcatatgtgattaattccaacgccgaatgtttcatgctcaagacctttaatcggcgccccgattgttccgtaaagcgagacagcgatccaatcgccttccgcttcactttcataaggatttcccctcaaaacggcaaacctcaatcccaccgtccgaagcagcgatcccagcagcatttcacctctggtcacgccatgcaaagcctccatcgtcgcatgataaagcgcatgtgactcccgataaccctcagattgaatgacaccgctctttttggaagcggtttcaattgcggctactactttatgtgcgtccattgatcctaccttgccaagacagaccttccatccgtctcgctccagctcctcaacctgcgtactttcttccgcctcattcagcagcaggagaacagacagccggccgatccgacgctctttatgcagtgtcatatgaatcactcaattcctaaaaattctgataactattaactgagtattatattaattggttcagcagcagaagtcaaaaggtttttttatagtctttaacaagttagattgctattgtaatagcgtgacgcagaaagcagaacaggttttttcagcgattgcacacgatatccagacaaggaggcaagcgccgctgtctaactctcaatatgcgtttactaagtcgtatttttcgcaaggcgttttataaagagccagccgaatgactctggtgttgacgggcaatcaggcatcatcttaaaaaacgccgacaacgaaatggctgtatcacagttgatgcaaaacctgacaaagcagttattacatgtacgcgaaagaaaaacagacgtgatgcaagaaggagaaacagcaaaagagttgaactatgaaggagaggatatgcaagcaacaagttctgcgcaaaacagacagacatcagtctgactatgtaagtgaagtgagaaatcacctatctggatgaatatgaaaacattcggctgttttaataggccggggtatcttcatagagaaatgtaagcgtttaaaatttaataaaaaagagaggcgaattgtttagatgttcaaccgattgttccgtgtatgttttcttgcagctcttatcatggccttcaccctcccaaactccgtctatgcacaaaaacctatatttaaagaagtcagcgtccatgacccttccatcattgaaacaaacggcactttttatgtttttggatctcatctcgcttcagctaaatcgaatgacctcatgcaatggcagcagctgaccaccagcgtaagcaatgacaacccacttatcccgaatgtctatgaagaattaaaagaaaccttcgaatgggcgcaatccgatactctttgggcggctgacgtcacgcagctggcggacggcaaatactacatgtactacaacgcctgccgcggcgattcgccaagatccgccatgggtgttgccgttgctgacaacatcgaaggcccatacaaaaacaaaggcatctttttgaaatcaggaatggaaggcacaagcagcgatggaacaccgtatgatgcaaccaaacatccgaatgtcgtcgacccgcatacctcttttgataaagacggcaagctgtggatggtgtacggatcatactcaggcggcattttcatacttgaaatgaatccgaaaacgggcttcccgcttcctggacagggatatgggaaaaaactgctcggcggcaaccacagcagaatcgaaggcccgtatgttctctacaatccagacacccaatactactacttatacctatcatatggcggtctcgatgcaacaggcggctacaacatccgtgtggcccgctccaagaaaccggacggcccttactatgatgcagaaggcaatccaatgctcgacgtccgcggcaagggaggcacattcttcgacgaccgttccatcgaaccatacggcgtcaaactcatgggcagctacacttttgaaacagaaaatgaaaaaggcaccgggtacgtctcaccaggccacaactccgcatactatgatgaaaaaaccgggcgttcctatttaatcttccacacccgcttcccgggcaggggtgaagaacacgaagtcagagtccaccaattgttcatgaacaaagacggctggccggtagcagcaccatatcgttatgcgggcgaaacattgaaagaagtaaaacaaaaagacatcacaggaacatacaaacttatccagcacggaaaagacatctcagccgacatcaaacaaaccatcaacatccagctcaacaaaaaccacaccatttccggggaaatgaccggaacatggaggaaaaccggaaaaaacaccgccgacatcacgttagcaggcaagaagtataacggggtatttttacgccagtgggattcggtgagagagaagaacgtcatgacgtttagtgtgctgaataccagcggtgaggctgtatggggatctaaataagatggagaagcgccttcgagggaaggtgtttttttatgagctttattgactataagaaacagttaagtgggaggaaaaattagaactggaggagagattaaaggcttaaataaaaagtccctactatgattgttttctcctttcatagggtgatgagatcgtatttttagcaatttagaaccagttctatacctctcaagacaatcctttttacctatttatccaatatgacccatcatgtaatatgaaaatagtctgtattgtaaagaatttacacagtttgatagaaacacgaggtgttgcggcatgcatagtgaaatgttgttacattcggtaaaagccgacttacatgaaaagcaggaacagatccatcaattaaaacgagtgctgcacgaaattaggcaaatcaaacacgatttctctgaggcccagcatctcattcaccggcctcatcttaaccgggaggcatggagaggaacacatgctgagcggtttgaagatattcgtgaaggaatgaacaaagcatatcagcaaatcaaaagcgatcaagtcagcggaatcatcgaaagcatagaagggaaaatccactcattagagggcgatgtgtattctataagacgccaaatcacgaggatagagcatgaaatagagaaggaaaaacataaaaagtgaggtgagcacaaatggcacaggaaattaaaatggtgtatgacacagtgaagcaagggctttctcagctcaagaattcagctgaactcaagtcctcattgcccggtcatctctcaggcagaaaccatttgaatgttgtgaagtccatcgagcaattaaataaggacatcaaagagctcactgaagcatatgcgtctgttctggccaagcatatcgcacaaacggaaagcgcggtaaacgccatgaaggaaacggacgaaaacatatcatcttccatgaaataaagcgcgggaggacaagggattgaaaacattagatgtccacgctcttcacgagggcattcagcatacgattgagaaactggacaagcaaaaacaacagctggagaagctggaaaaaagcgttgagcatctggcaggcatgaaggatgcgctgaaaggaaaaggcggagatgccatccggaccttttacgaggagtgccacaagccttttctccttttctttggcatatttatcgacgaatacaaaaaagtgctgaaacaaacacagcatgcgatttcctctgtagaatctaactcccacggcatgatcgcagaggcttttctctcacacgatgcgagacatggggtcaagcatgcacgagaagtgacagagcagctcactgacgcagtcaatcgccagacatcagccatagatcacatcgtcagcctgccgacagtcaatgattccttttttcggatggaaacagaacaggctgagcggctgatttcagacaccctgaataagctctttcaatttgacggccagcaaacccaagcactagaagccggaaaatcagattttcaaacgatgaaaaaatacattgatcagctcgaaaccatgtacaccggcccgaaaattgaaatcacaggctacaaaagcggctccatcctgaaatcacaggaagaagaaaacatcaaccaaatcttcggcgcgattaacccgcaaatgaagcaggcggatgattcaccgatggagatgatgctgaagaaattagccgagaatgaaaagtctaaagtggattcagttgtcaaaacgggtgattctaaaaaggtaagtaaaaatatcatcgttatcaatggtaaagtgtataatacgagtgaacatagagaacatataaaacctgatttctcaaatgcagaggttaagcaagtcgtttataatgatacactttacaatgtatacatatctggtaatgacatgaagcttgaacctgtcgtctcgctttcggacattaaagtggatgagaatggatatgtgaaaattttagagacggctgtagaacttaccggcgtgtatgatctatttaaagcagccacgggcagagatccggtatcaggcgaaaaagtcacagggaaagaccgtgttgttgcctccataaactcagtaccatttgccaaaatagctaagttagaaaagttaatagatattaataaacttattaataatggggaaaaggctaagaaggcctcggaagttaaaaacgttgctaaggataaagggaaaattgcgaatgatgtaagtggatctgctaataaaattaattctgatttaataaaaaagtatgctagagatatagaacaacgcacaggtagagaattacctaaaaatcaaatagataaattaaaggaagcattaagaaataaagaatataaaaaaatgtcaccaatagagactgcaaaacacaggactaaatttgataaagtaaaaaataaagttataaaagaatgggaagaaaacactggacaaaaatggcctgtttataaggaaaatgttgtatctgaaaaaacaggtaaaattattagaaaaaaaggggataagtatgatgctcaccatataattgaaaatacttttggcggaaaacatgaatggtggaatatgcatccagcaaaatttcctaacgagcatcaagctgggattcatggtacaggctcaccagcaaatgaattatttaaaggaggcaaaaaaaaatgagttataattttataaaatcaaacaaagaaaatgatttttatccagtgaatcaaagtgagattgaagaggttgaaaaaaatttaaacttaaaattacctagtgaattagtgaatttttatttagaagttggctatgggtttattaaaggatcagagtttaatactaatcgcattttggatccatattctgtaagagactttcgattgaggataaatgactttgaattttatcctgacatagaaatatatgatgagtttgagaatgataaattaatattttttgaaggtagtgaatcggcattaatgtcaattgaattaaatgataataataaaaatccgatttactattatgatattcaaattgcaacttctcttaccgagttcttaagaaaaatagaagagaatgatcagtattatcttgatttattagatgatgaatgattttaacattatcccgttacctctcccttaaaggagcaagatgacatgttattgatcaataaacagaaggaccctgtttttcagtttttagctggaacattccatcaagatattgaaactcctgatgacgctatacaagagttattaatagaggaaagtaaggaatatttggaggatgctattgtctttttaacggattttattgaaagtgagcattcagacaataagaaaaacgattacattcaatcttgcgcagatggcgtgtatcttcctgcgtttaatttagaaccaatagattggctaaagaatgtaatagtacagataaagaagtctttaaaaaaatttaaacggtaacgattcataaccttgattggaaaaaatgcctttcaaggtttttaattacaataattttttattgaagttaatactaagttcaaatctttatgattacttttgttctagaaacgatagtcaacaccaaaaatgaaagcgttgacatctcacgaatctagtgctaaagtatacctacaaacaaataaaacgacccgtcaggattgttactgcgaaagcaggcaaaacctaaatggtgcaggtgcaggaggagactctcgcaatctgtgtcatttaggtttttttattctcttttaggaggtgatgcagcatttgatacaaaaaaagctggtgaaaggcggccacctttcatccagcagtccccccataaaaaggaggtatacacatggattatgataaattatcgaaggacatattacaactcgtaggcggtgaagaaaacgttcagcgcgtgatccactgcatgacgaggctgcgttttaatcttcatgacaacgcgaaggcggatcgcagtcagctggagcagctgcctggagtgatgggcaccaatatcagcggcgagcagtttcaaatcattatcggaaacgatgtgccgaaggtgtatcaggcgattgtgcggcacagcaatctcagtgatgaaaagagcgctggttcatcctctcagaaaaagaatgtgctgagtgcggtctttgatgtgatttctggggtgtttacccctattctgcctgcgattgcgggagcggggatgatcaaaggacttgtggcgctggcagtcacgtttggctggatggcggagaagagccaggttcatgtcattttgacggctgtcggtgacggtgcgttctacttcctgccgctcctgctagcgatgagtgcggcgagaaaattcggaagcaatccgtacgtagcggctgccattgcggcggcgatcctgcatccggatttgacagccctgctcggtgcggggaaaccgatttcctttatcgggcttcctgtaaccgctgccacttattcgtcaacggtcatcccgattttgctgtcgatttggattgcttcatacgtggaaaaatggattgaccgttttacacacgcatctctcaaattgattgtggttccgacattcacgctattgattgtcgtgccgctgacattgattacagtcggtccgcttggcgctattttaggagaatacttgtcttctggggtcaattatttgtttgatcatgcagggcttgtggcaatgattttcctggcgggtacattctctttaatcattatgacgggcatgcactatgcctttgtgccgatcatgatcaacaacatcgctcaaaacggccacgattatttactgccggctatgtttttggcgaatatggggcaggcgggagcatcatttgccgtcttccttcgctctagaaacaaaaaatttaaatcactcgcgcttaccacaagcatcacggcgctgatggggatcacagaacctgcgatgtacggcgtgaatatgcgattgaaaaagccgtttgcggccgctttgattggcggtgcagccggtggcgcgttttacggcatgacgggtgttgcttcctatatcgtcggggggaatgcaggtctgccgagcatccctgtctttatcggcccaacgtttatttacgcgatgatcggccttgtgattgcgtttgcggcgggaacatcagctgcgtatttgcttggattcgaggatgtgccttctcaccgcagccagcagccggcagtgcatgaaggcagcagagagatcattcacagcccgattaagggagaagtgaaagccttaagtgaagtcaaagacggagtgttttctgctggggtcatgggaaaaggatttgccattgagcctgaagaaggagaagttgtttcgcctgttcgtggaagcgttaccaccatttttaaaacaaaacacgcaattggcattacgagtgatcagggagctgaaatactcatacacattggattggacacggtaaagctggagggacaatggttcacggctcacatgaaagaaagcgacaaggtcgcaccgggagatccgctcgtgtcctttgatctggagcaaatcaaagccgcgggatatgacgtcattaccccggtgattgtgaccaacacagaccaatattcgttttcgccggtgaaagagatcggtaaagtgcagccaaaagaagcgctgcttgctttatcttgaaaaaactaatggggtgatcaatatgagttcaaatgaaaaacgatttccagaaggatttttatggggcggcgcagttgctgccaaccaagtggagggtgcttataacgagggtggtaaggggctttcgacagctgacgtatcgccgaacgggatcatgtctccatttgatgaatcaatgacttccttgaatctgtatcacaacgggattgacttttatcatcgttataaagaggatatcgccttatttgcagaaatgggatttaaggcgttccgcacatcgattgcgtggacgagaatttttccgaatggcgatgaagaggagcccaatgaagaaggcctcagattttatgatgatctgtttgatgagctgttaaagcatcatattgagcctgtcgtaaccatctctcattatgagatgccgctcggtttagtgaaaaattatggcggctggaagaatcgcaaagtcatagagttttatgaacgctatgccaaaacggttttcaaacgctatcaacacaaagtgaagtattggatgacgtttaatgaaattaacgtagtgctccatgcgccatttaccggaggcggtcttgtttttgaagaaggagaaaacaaattaaacgcgatgtaccaggcggcacaccaccaatttgtggccagtgctcttgctgtcaaagcgggtcacgacatcattcctgattcgaaaatcggctgtatgatagcggcaacgacaacctatccgatgacttctaagccggaggatgtcttcgcggcaatggagaatgagcgcaaaacacttttcttctcagatgttcaggcaagaggcgcatacccgggatatatgaaacgctatctggcagaaaacaatattgaaattgaaatggctgaaggcgatgaagagctcttgaaagaacatacggtggattatattggatttagctactacatgtcgatggcggcgagcacagatccggaagagcttgcaaaatcagggggcaacctgctgggcggagtcaaaaacccttacctcaaatcatcagaatggggctggcagattgatccgaaaggcttgcgcatcacgctcaacaccttatacgaccgttaccagaagccgctgttcatcgttgaaaacggccttggcgctgtagacaaggttgaagaggacggcacgattcaggacgattacagaatcaactatctgcgtgatcatttaattgaagcgcgcgaagccattgcggacggcgttgaattaatcggatacacatcatgggggccaattgaccttgtcagcgcatctactgcggaaatgaaaaagcgctacggcttcatttatgtagaccgggacaatgaaggaaatggaacatttaaccgcatcaagaaaaaaagcttcaactggtatcagcaggttatcgccacaaacggagagagtctctgacaattttttgaaaactcatgcgcttcaattgacaataacgaaatgcaggcggacaataaaagagaaagatgaaccacccacagtccgaaaggcgggaagagcatgtttaacaaaatgttagtagcgattgacggatcagacatgagtgcaaaagcgcttgatgccgcagtgcatttggcaaaagagcaacaagcggaactaagcattcttcatgtggggagagaagccgtcgtcacgacttcttctctgacgggaattgtctatgtgcctgaacactttattgatgaaatcaggaacgaggttaaaaaagagggcctgaaaatccttgagaatgcaaaagaaaaagcagccgaaaaaggcgttcaagctgaaaccatttacgcgaatggcgagccggcgcatgagatactaaatcacgcaaaagagaaaggcgtcagcctgattgtagttggcagccgggggatcagcggcctgaaagaaatgatgcttggaagcgtcagccataaagtgtctcaattatcaacatgcccggttttgattgttcgatagatttgtaaaaaaagcgcccttgggcgcttttttttatttagaatagaagtgttataatatctacatgtaaaaaagaggaattctatgtgtagatttctgaattcacaaaaaacagtttatgctatgcagtattggaggtagaatacgtttgatgcaacaggatccttccatatcgtcaaaacaaaaatcaacagccgtaatcaaaatggtcatctctatggtgattttcggctccatcggctttttctcagagcataccaatctgccgtcatttgaattggtctttgtccgctgcctttgcgcgacgctgtttttaggcttttgctggctggcgtccggccagtataaaactgaaaaatggagcaagagagacgtgctgcaaacattggcgtgcggtttctttcttgtattcaactgggtgttcttatttaagtcttttgaagaaacgtccgttacaattgccatctctgtttatcatctagcgccggtgcttgttcttcttctggggagcttcttctacagagagaaattaaatgtgatctccgtcagctccattatcatctgctttcttgggactgcgctgatttccgggattaacggcagcacatcattgacacagctgatgggatcagggatcatatgggcagttctcgccgcactgttttatgcgttcaccactttattgggaaaaggcattcacaatctcagtccttacacgaccaccttcttgcagacaggtttaggggttatcatcctgattccgtttattcactttggcgcttttgcggacctatctcagggaaactggattatggtggtatctaccggcatcatccatacgggtattgtatatttgctgttttttgacagtttacgatttttatcaacgaaatttatttcaatcattgtatttctcgaccccgctgtcgcgatcgtgctcgataccgtcttcacaggcttccgccctgacctctatcaaacgcttggcatcgtaatgatctttgcgggcatggccttgacgcttgtcaggaggcaggggaaggcgaatgtgacagctgagggtacggatattgaacaaatacaataaaaaatgtaaaaaggcctatgcggcctttttttgttttaggtcaattgactctcgctaatccttaaaataagataaattttctagaaaaatattgtaatgatatttcagtctagttaagattattgagtaaatattacttttattacaaaaggagagaggaaatgaaaaaaagaaagaggcgaaactttaaaaggttcattgcagcatttttagtgttggctttaatgatttcattagtgccagccgatgtactagcaaaatctacagaagaagagaatggaaaccgtattgctgccgatgatccagaagaaactcttcagaaagaacaaactgaggaagctgtaccttttgatccaaaagatataaacaaagagggtgagatcacctctgaaagaacagaaaatacaaaactctattatgaaggtgacggtgtctataaacaggaagtataccttgatcctattcatacaaaggaaacaccggatgccgactgggaagacatttctcctgagttaaaagagtcgacaagcaaacaagtcgagacagagaacgctattttgaattcagattttcaaaagcaaatgaagaacgggctttatgcgacttttgagcataatgaccataaggttacatattcactagcagaagcgaaaggcccgaataaaacttcacttactccgaaagatacctcagcagattataagactgacagtaatgagattgtgtatccggatgtgtttccgaatattgatcttcagactttcacattcaatgaaaacataaaagaagatttagtccttcatcagtataatggatacaacacatttacatttcagttaaaaaccgatttgcaggctaaagaacaagaggatggatccattgatttttctgatgaaaaaggaaaagttgttttttctgtgcctaagccttttatgacggattcaaaactagatgagctttccggcgaggttgaacggtcagacaaagtcagctataagctggaaaagaatgaagaagggtatttgcttcatcttacggcagacgagaactggctgaaagacccagaacgcgtatatccagtatctatcgacccgtcaacttctttatctgtttcatcggatacgtttgtcatgagtgcctacccgacgacgaactattcggcctcctcacaaaaatgggatgctaatttaaaggcctatgtactgaaaacgggctattatgacaaaacaacaggcacaaactatgcgttcatgaaatttaacaacctaaagccaattcaaaatatgactgtcactaaagctacattaaaaacatacgtagcccattcctattatggaacaaaggcaaccggcctttggctggatacggtcaacagcaattatgataatgcaaaagtgacatggaacaccaaaccggcatctaaaaatatcggaaaagccgacgtccataaaggacagtgggcgagttatgatgtgaccgctgctgtaaagtcatggaactccggcggggccaactatggatttaagcttcatacaaacggaaacggcaaggaatattggaaaaaactaatttcttcagcgaactccgccaataaaccatatattgaagtgacgtataccattccaaagggaaacacacctacaatcaaagcctatcacaacggcgattccactggttatttcgatatcagctggaaaaaggttgaaggcgcaaaaggatataaggtatggatttacaatggtaaggaatatcaagcgatttctgcaggcaacgtcacgtcgtggagcacaaaaggtaaaaaaatctggcctacgagcgcagaaattgcctccaagagatataaactgcatctggacggcaaggatggagctgaattggcattagatccatccccggtctataagaattccggcggaagctatgctacaagcaaaaactattggattggcgtcagtgcgatatttgaccaaggtgaaggagcgatgtccgcaccggcaaagcccgttatccctaatgtaggaaaagcacaagcaccgtcagcaaagggctacaataatgggaatgccacaggatacttcgacctttcttggaaagctgtatccggtgcaaccggctataaggttcaggtgttcaatgggaaaggctttgagacacttgatctcggaaatcagacgtcttggaccacaaaagggaaaaagatctggccgacaagtgcagaaatcaaggcgggaaaatatgctcttcacctaaaggacggaagcggagcagagctgccgatcaatcccggaccaacctataaaaacgccgggggagatggagccaaaagaaattactcgtttaaaattatcgcatacaacaaagacggcgaagccattgcatccccggctgctaccccggcacttcctgatatcgctaggccaaagaatgtaactggctatttgtatacaaatacaaaatcgagtcaaacgggttatgtgaatttgatatgggaaaaggttcaaaatgcgaagggctataaagttaacatttacaacggtaaagaatatcagtcctttgatgttggtgatgctgatcattggacaacccaaaataaaaacatctggccgacttctgaggaaatcaaagccggaagctataagcttcatacagatggaaaaggcggggaattagccctcgatccatcacctgtctataacaatgcaaatgggaattacaaagggaagaagaattattctttcacgcttgtcgcctatgatgcgaatggtgaaacgattccaacggcgccctttaacccaacgttccatgaaggcgcagaattcctaggtacagaagagtactggtctatcattgatatcccaagcggccagttaaatggtgcgacaggcaatgtcattgtgaatgaagaagatttgtcaattgatggacgcggtccgggacttggcttatcgagaacctacaacagtcttgacagctctgatcacttatttggacaaggctggtatgctgatgcagaaacatctgtcatctcaacggatggcggggcaatgtatatcgatgaagacgctacgacacatcgattcacgaaaaaagccgatggcacgtatcagccgccgaccggtgtatatcttgaattaacagaaacagctgatcagttcatattaaaaacaaaggatcaaaccaacgcttatttcaataaaaaaggcggcaaactccaaaaggtagtggatggccataacaatgcaactgtctatacttacaatgacaaaaatcaactgaccgccattacagatgcatcaggccgcaagcttacatttacctatgatgaaaacggccatgtgacgtccatcacaggacctaagaataagaaagtcacctactcatatgagaatgatttgctgaagaaggttacagatacagacgggactgtcacaagctatgactacgatagtgaagggcgccttgtcaaacaatattcagctaacagtaccgaagcaaagcctgtctttaccgaatatcagtatagcggtcaccgtctcgaaaaagcgatcaacgctaaaaaagaaacatatgtctacagctatgatgctgataaaaagacgcttctcatgacacagccaaatggccggaaagtacagtatggctataatgaagcgggaaatccgattcaggtcattgatgatgcggaagggttaaaaattacaacgaatacaaagtatgaaggcaacaatgttgtagaagatgtagatccaaatgacgtcggcaccggaaaagcaacggaaagctatcaatatgacaaagatggcaacgttacgtcggttaaagatgcatatggaactgagacatacgaatacaacaaaaacaacgatgtcacaaagatgaaggataccgagggcaatgtcacggatattgcttatgacggactggatgctgtatccgaaaccgatcagagcggaaaatcatcgtcagcagctgtttatgataaatatggaaaccagattcaatcgagcaaagatttatcagcttcaactaatattttgaaagatggaagctttgaagctcaaaaatccggctggaatctgactgcctctaaagacaggcgcaaaatttcagtcatcgccgataaaagcggagttctttccggatcaaaggcattggaggtcttgagccaatcaacgtctgccggaacagatcatgggtattcgtcagcaacacaaacagttgagctggagccgaatacaacctatacattaagcgggaaaatcaaaacagatcttgcgaaatcaagagcctattttaacattgatttgcgagacaaagatcaaaaacgaattcaatggattcacaatgaatacagtgcattagccggaaaaaatgactggacaaaacggcaaatcacttttacgactccagcgaatgcaggcaaagctgttgtgtatatggaagtcgatcataaagataaagatggcaaaggaaaagcatggtttgatgaagtccagctggaaaaaggcgaagtatcatcaagctataacccagttcaaaacagcagcttcacatcagcaacggaaaactggaatgtaagcggagcatccgttgattctgaagaaggctttaatgatgatgtatcattaaaagctgcccggaccagtgcgtcccaagccggatcagtaacaaaacaaaccgttgtcttagggcaaagcgcaaatgacaaaccggtttatctcacactgacaggaatgtcgaaagcaagcagcgtcaaatttacagatgaaaaagactattctctgcaggcgaatgtcacttacgctgacggcagcacaggcatctacaatgcgaaattcccttctggaacacaggaatggaaccgagcagctgtcgtcatccctaaaacaaagccgatcaataaagtcgatatcagtattctgttccaaaagagtgcgacaggcacagtctggtttgatgatatccgtttgattgaaggaagccttctgactaaaagcacgtatgacagtaatggcaactatgtgaccaaggaagaggacgaactaggttacgccacttcaactgattacgatgaaactggtaagaaaacgtctgaaacagatgcaaaaggtgaaaaaacaacctatacgtatgatcaggcagaccaattgacaaacatgacgctctctaacggcacgtctatccttcacagctatgataaggaaggcaatgaggtaagcaaaaccatccgggcaggagcagatcaaacctataaattcgaatatgatgtcatgggcaagcttgtcaaaacaactgaccctctcggcaatgtgttagcaagcgaatatgatgccaacagcaacctgaccaaaaccatttcaccaaatggcaacgaagtgtctctttcttatgatggaacagaccgggtgaaatcaaagtcgtataacggtacagaaaagtacattttcacgtatgacaaaaatggaaatgaaacgtcggtcgtcaataaagagcagaacaccacaaagaaacggacatttgacaacaaaaaccgtttaaccgaactgacagaccgcggcggcagccaaacttggacatatcctagtgactccgataagctgaaaaccttctcgtggattcatggggaccaaaaaggaacgaatcaatttacgtataacaagctggatcaaatgattgagatgaaagacagtacatcctcatattcatttgattatgatgaaaatggaaacgtccaaacctttattacgggcaacggcggcggaacaagtttttcatatgacgaaagaaaccttgtaagctcgctgcatatcggtgacaaaaacggcggagacattctgacggaaagctatgaatatgatgccaacggcaaccgcacaacgataaacagctcagcaagcggcaaggtgcaatatgagtatgggaagctgaatcagcttgtcaaagaaacccatgaagacggtactgttattgaatacacatatgatggattcggaaaccggaaaaccgttacaactataaaagacggctcaagcaaaacggtgaacgcttccttcaacatcatgaaccagctgacaaaagtcaatgatgaaagcatctcttacgataaaaacggcaaccgcacatccgacggcaaattcacatatacgtgggatgcagaagataacctgaccgccgttaccaaaaaaggcgaagacaagccattcgcaacatataagtatgacgaaaaaggaaacagaatccaaaaaaccgtcaacggaaaagtcacgaactacttctacgacggagacagcttgaacgtcttgtatgaaacagacgcggacaacaacgtcacaaaatcatacacgtacggagacagcggccagctgttatcctacacagaaaatggtaagaaatatttctatcactacaacgctcacggcgacatcatcgcgatctcagacagcactggaaaaaccgttgccaagtatcaatacgacgcatggggaaatccaacaaaaaccgaagcaagcgacgaagtaaaagacaatcgctaccgctacgcaggctaccaatacgacgaagaaaccggcctgtactatctcatggcccgctactacgagccaagaaacggcgtgttcctatcgctcgacccagacccgggcagcgacggagattcattggatcagaatgggtatgcttatggaaataataacccagtgatgaatgttgatccggacgggcattgggtatggcttgtggtaaatgccggatttgcagcctatgatggatataaggcatataaatcaggtaaaggatggaaaggtgctgcttgggcagctgcttctaattttggtcctgggaagatatttaagggtgctagtcgcgcctataagtttacgaagaaggcagttaaaatcacaggtcatacaagacatggacttaatcaatctataggaagaaatggaggccgtggagtcaatttaagggccaaactgaatgctgtgcgaagccctaaaaaagtaataaaacaacctaatggggcaacgaaatatgttggaaaaaaagctacagttgttttaaataaaaggggtaaagtaatcacagcttatggaagttcaagagctaagggttctaaacacgtattccatacacacggaaaaggaaataaatctaagagaaggcgttaataaggttaagcgagggggggatgacaactaccctcacttaaactttaaatgaggaggaaatatggccaaaataaaagatgattgtatagaacttgaattaacaccgagaaggtatcaagagttggacgatgatccatttattttatctgtatttgaattgttggaaaataagaaagccgtcgttcgcgatttttctgctgttttattagaaagtgaatataaggtgttgatatctgggatcgaaactatgataaaaggaaatcaagacagtatcagtttagagactattgaaccattcttatttcttagtattgatcaagaaaacggaaattacagaattaagattaaaattatatttgatgattataaagaaagtaagtcgaactccaacttgttcgaaattaattgtaatgaagaaaagctagagtcttttgtgaccgctttaaaattaaatcttgaaaatacaaaaaatccttctaaacttccttaattataaataatttctgcattggataaaaatggggcatttattgatggaacattaaataagagatgttaccatcctctcttatttgtatgacaaaagaatctaaaaatatagaattgattgggatgaagaggatttgccaaaaaggttcccagcgttttgtgaaaagcccactgggtgagttttaagcagttgaagataaagcttgtatcgataagcgatacaagcttttttagaacaaatctaaacatgaacgacaacgaaaacaagagaatgatgaatcaatttaaaagaagttgagaaattgacagcggagggaatgcggctcatgcaaaaaagattgatcgaaaaactcgccgagaataaaagacgtttattgatgagcgaaatcaaagaaaaactagtcccttgtgcagaaagaggcttcacttatcgttttgctgatctggcgcaaagcaggcaattgcttgagctggttttatcaaattcaataccagccaacacccgtgaggttgatgccctcgaaaaaacggaagcgaaacagctgatctggaaaatatctcagtcatatgttgcttacgatgaccgggacgttctgctgtttcatcaatacagcagcgaaattggtgcgttagtttgttcttttggaaaatgtctcgagcaccttgactgcttattggagtgtattgagttcgatgaagggattctcaatcatagttttattttggttgagcctaagtgccagtttggtttatgtatattgcacacggaatacggatgtgagcttgtttattggtagattggaaaccttttggaacatatcttttacggaaaaagcttcaatatctaaatatcagtacggtgctttgcatactaataaaaaatcatttagtacttgaatacgtggtgatcaaattgagcgagacaaatctaatagaatgcataaataaaatcaaaagtgtcttaaatggacaaacaacaagagaagaagtgtcggattgggctggaacttatgtttatgcggatgaccccgaagtagaagacgatagagtctgggatatgttaatccttctaagtgggattgatttgaaagattcatcagaaacttatttgcattcaacagatgatttaaatgattggatcaaacaatatacggagtaatttgttttctgcttggtggcaaggcgttattgtttaaaaagaggcaggggatgacaatgtatcaaacgattaatgaatgggttgattatatagataaggggtgcagtgtccttcatttagattttaatgtgtttaaaaaagaactctcacttgatattaaggtttttgaagatgaaggtgaatatacgcataaaatttcatttcaaaatgtggcatccgcttattatagtgcagatgttggcgacatgagattggaaaaaatagatccggaagaatacaattggcaagtatttgagatgagttatcatccagaaggaatcgggaatctatcaaattctataattccggagtatcaatcaaatgctaactttcttattgacatgaacagaatgctgattgctatagaagctgaaacagttcgctttgatgatcaatcgttttatgcataccaattaaacactaaatgatttaaggctgaattggaaagtagatttatcccaaaacgattaatgaaactaggttgtccgttactaatagctaataaatggtttattcttatcatttcatttcgaacctaggagcataaccaatgaaaaaattaaaattgaataaaatcatcaacgagaacacccaagattgttttttccatgctgatccacaggggcgtgtctacattggaaaagggttgaaaggtggtatcaccattacaatctatgatccttccggtgatgttcgggattttagagtgaaagagcagatttcatacagtgatattctgctctttcaacaatgtgcagatggctatgtcttcgtttattacgaatcgtacgagccgaaggtaaaggttttttcagaagagggaagggtgaaaagtgtttttcacttgccttcaggggtttcctgctgtcttttggattagaaacaacagctttgggtcggtttatgtgatgaagggatttatcatgatgagaatcccaacggccatagtgtgtggtgttttacgttagatggtcagcagaaggaaatacacattgatagaaagcttgaagaaatggatgcgcctgctgtagatgattgttatggacttgcagaaaaaaacggcttgatttatatgctgtattacggagatgcagtcattgccgcatttgatgaaacggtcgtgagacgggtgtggattctgtcggataaagagccggacttagaagcatttgatcagctcgcgatatccgaagaaggttttttggttgggacgttcaattgttacagtgcagaccttaagtcgtctctttatttgatttctgccgatgtgagtcaagagatggaagagataacatgctgtgattcgaacggtgaaggcctagatgttcaacagctgaaactgacaagttacgctgtttacgcagtggcctcttctggtgtttataagcaggatatccaataaggtgtagggatgagattatgatgaattggcgcgctttaagtcagacaaaacaagaccgcatctggtcagaagtgaacaagatc

SEQ ID NO: 3 - DNA, 20 bp, synthetic construct
  source 1..20: mol_type = other DNA
agagtttgatcctggctcag

SEQ ID NO: 4 - DNA, 15 bp, synthetic construct
  source 1..15: mol_type = other DNA
ctgctgcctyccgta